European Patent Specification EP 4 284 843 B1, published August 20, 2025. Title: NOVEL SIALOSIDES AND THEIR USE IN THERAPY. Applicant: CNRS ENS de Lyon INSERM UCBL. The sequence listing filed with the application follows.

SEQUENCE LISTING (2 sequences)

SEQ ID NO: 1 - DNA, 55 bp, Artificial Sequence
  Oligonucleotide comprising a SalI site
ggtcgacggtaaggagatatacatatgatttctgtttatatcatttctttaaaag

SEQ ID NO: 2 - DNA, 33 bp, Artificial Sequence
  Oligonucleotide comprising a PstI site
ctgcagttaaacctctttaggggtttttaaagg